European Patent Application EP 4 592 319 A1, published July 30, 2025. Title: ANTIBODIES CAPABLE OF SPECIFICALLY BINDING TL1A AND USE THEREOF. Applicant: FUTUREGEN BIOPHARMACEUTICAL (BEIJING) CO., LTD. Application EP. The sequence listing filed with the application follows.

SEQUENCE LISTING (68 sequences)

SEQ ID NO: 1 - protein, 107 aa, synthetic construct
DIQLTQSPGTLSLSPGERATLSCRASQSVSNHLAWYQQKPGQAPRLLIYGASKRATGIPDRFSGSGSGTDFTLTISRLEPEDFAVYYCQQYADAPLTFGQGTKVEIK

SEQ ID NO: 2 - protein, 117 aa, synthetic construct
ELQLQESGPGLVKPSETLSLTCAVSGLSFTDFYWAWIRQPPGKGLEWIGEINHKGNTSYNPSLKSRVTVSIDTSKNQFSLKLSSVTAADTAVYFCARDFPNYTFDFWGQGTLVTVSS

SEQ ID NO: 3 - protein, 107 aa, synthetic construct
AIQMTQSPGTLSLSPGERATLSCRASQSVSSHLAWYQQKPGQAPRLLIYGASRRATGIPARFSGSGSGTDFTLTISRLEPEDFAVYYCQQYADSPLTFGQGTKVEIK

SEQ ID NO: 4 - protein, 117 aa, synthetic construct
EVQLQESGPGLVKPSETLSLTCAVSGVSYSDYHWAWIRQPPGKGLEWIGDINHKGKTNYNPSLKSRVTISVDTSKNQFSLKLSSVTAADTAVYYCARDYPNFLFDYWGQGTLVTVSS

SEQ ID NO: 5 - protein, 107 aa, synthetic construct
DIQMTQSPATLSLSPGERATLSCRASQSVSTYLAWYQQKPGQAPRLLIYGASRRATGIPARFSGSGSGTDFTLTISSLQSEDFAVYYCQQYGDTPLTFGQGTKVEIK

SEQ ID NO: 6 - protein, 117 aa, synthetic construct
ELQLQESGPGLVKPSETLSLTCAVSGISFNDFHWAWIRQPPGKGLEWIGDINHRGHTSYNPSLKSRVTVSVDTSKNQFSLKLSSVTAADTAVYYCARDYPNFTFDLWGQGTLVTVSS

SEQ ID NO: 7 - protein, 107 aa, synthetic construct
DIQLTQSPGTLSLSPGERATLSCRASQSVSSYLAWYQQKPGQAPRLLIYGASKRATGIPDRFSGSGSGTDFTLTISRLEPEDFAVYYCQQYGDSPLTFGQGTKVEIK

SEQ ID NO: 8 - protein, 117 aa, synthetic construct
ELQLQESGPGLVKPSETLSLTCAVSGVSFSDYHWAWIRQPPGKGLEWIGDINHRGHTNYNPSLKSRVTVSIDTSKNQFSLKLSSVTAADTAVYFCARDFPNFIFDYWGQGTLVTVSS

SEQ ID NO: 9 - protein, 107 aa, synthetic construct
DIQLTQSPGTLSLSPGERATLSCRASQSVSTYLAWYQQKPGQAPRLLIYGASKRATGIPDRFSGSGSGTDFTLTISRLEPEDFAVYYCQQYGDSPLTFGQGTKVEIK

SEQ ID NO: 10 - protein, 117 aa, synthetic construct
ELQLQESGPGLVKPSETLSLTCAVSGVSFSDYHWAWIRQPPGKGLEWIGDINHRGHTNYNPSLKSRVTVSIDTSKNQFSLKLSSVTAADTAVYFCARDFPNFIFDFWGQGTLVTVSS

SEQ ID NO: 11 - protein, 107 aa, synthetic construct
DIQLTQSPGTLSLSPGERATLSCRASQSVSNYLAWYQQKPGQAPRLLIYGASRRATGIPARFSGSGSGTDFTLTISSLEPEDFAVYYCQQYAASPLTFGQGTKVEIK

SEQ ID NO: 12 - protein, 117 aa, synthetic construct
ELQLQESGPGLVKPSETLSLTCAVSGVSFTDYHWAWIRQPPGKGLEWIGDINHRGHTNYNPSLKSRVTVSIDTSKNQFSLKLSSVTAADTAVYYCARDYPNFIYDYWGQGTLVTVSS

SEQ ID NO: 13 - protein, 11 aa, synthetic construct
RASQSVSNHLA

SEQ ID NO: 14 - protein, 7 aa, synthetic construct
GASKRAT

SEQ ID NO: 15 - protein, 9 aa, synthetic construct
QQYADAPLT

SEQ ID NO: 16 - protein, 5 aa, synthetic construct
DFYWA

SEQ ID NO: 17 - protein, 16 aa, synthetic construct
EINHKGNTSYNPSLKS

SEQ ID NO: 18 - protein, 9 aa, synthetic construct
DFPNYTFDF

SEQ ID NO: 19 - protein, 11 aa, synthetic construct
RASQSVSSHLA

SEQ ID NO: 20 - protein, 7 aa, synthetic construct
GASRRAT

SEQ ID NO: 21 - protein, 9 aa, synthetic construct
QQYADSPLT

SEQ ID NO: 22 - protein, 5 aa, synthetic construct
DYHWA

SEQ ID NO: 23 - protein, 16 aa, synthetic construct
DINHKGKTNYNPSLKS

SEQ ID NO: 24 - protein, 9 aa, synthetic construct
DYPNFLFDY

SEQ ID NO: 25 - protein, 11 aa, synthetic construct
RASQSVSTYLA

SEQ ID NO: 26 - protein, 7 aa, synthetic construct
GASRRAT

SEQ ID NO: 27 - protein, 9 aa, synthetic construct
QQYGDTPLT

SEQ ID NO: 28 - protein, 5 aa, synthetic construct
DFHWA

SEQ ID NO: 29 - protein, 16 aa, synthetic construct
DINHRGHTSYNPSLKS

SEQ ID NO: 30 - protein, 9 aa, synthetic construct
DYPNFTFDL

SEQ ID NO: 31 - protein, 11 aa, synthetic construct
RASQSVSSYLA

SEQ ID NO: 32 - protein, 7 aa, synthetic construct
GASKRAT

SEQ ID NO: 33 - protein, 9 aa, synthetic construct
QQYGDSPLT

SEQ ID NO: 34 - protein, 5 aa, synthetic construct
DYHWA

SEQ ID NO: 35 - protein, 16 aa, synthetic construct
DINHRGHTNYNPSLKS

SEQ ID NO: 36 - protein, 9 aa, synthetic construct
DFPNFIFDY

SEQ ID NO: 37 - protein, 11 aa, synthetic construct
RASQSVSTYLA

SEQ ID NO: 38 - protein, 7 aa, synthetic construct
GASKRAT

SEQ ID NO: 39 - protein, 9 aa, synthetic construct
QQYGDSPLT

SEQ ID NO: 40 - protein, 5 aa, synthetic construct
DYHWA

SEQ ID NO: 41 - protein, 16 aa, synthetic construct
DINHRGHTNYNPSLKS

SEQ ID NO: 42 - protein, 9 aa, synthetic construct
DFPNFIFDF

SEQ ID NO: 43 - protein, 11 aa, synthetic construct
RASQSVSNYLA

SEQ ID NO: 44 - protein, 7 aa, synthetic construct
GASRRAT

SEQ ID NO: 45 - protein, 9 aa, synthetic construct
QQYAASPLT

SEQ ID NO: 46 - protein, 5 aa, synthetic construct
DYHWA

SEQ ID NO: 47 - protein, 16 aa, synthetic construct
DINHRGHTNYNPSLKS

SEQ ID NO: 48 - protein, 9 aa, synthetic construct
DYPNFIYDY

SEQ ID NO: 49 - protein, 214 aa, synthetic construct
DIQLTQSPGTLSLSPGERATLSCRASQSVSNHLAWYQQKPGQAPRLLIYGASKRATGIPDRFSGSGSGTDFTLTISRLEPEDFAVYYCQQYADAPLTFGQGTKVEIKRTVAAPSVFIFPPSDEQLKSGTASVVCLLNNFYPREAKVQWKVDNALQSGNSQESVTEQDSKDSTYSLSSTLTLSKADYEKHKVYACEVTHQGLSSPVTKSFNRGEC

SEQ ID NO: 50 - protein, 446 aa, synthetic construct
ELQLQESGPGLVKPSETLSLTCAVSGLSFTDFYWAWIRQPPGKGLEWIGEINHKGNTSYNPSLKSRVTVSIDTSKNQFSLKLSSVTAADTAVYFCARDFPNYTFDFWGQGTLVTVSSASTKGPSVFPLAPSSKSTSGGTAALGCLVKDYFPEPVTVSWNSGALTSGVHTFPAVLQSSGLYSLSSVVTVPSSSLGTQTYICNVNHKPSNTKVDKKVEPKSCDKTHTCPPCPAPEAAGGPSVFLFPPKPKDTLMISRTPEVTCVVVDVSHEDPEVKFNWYVDGVEVHNAKTKPREEQYNSTYRVVSVLTVLHQDWLNGKEYKCKVSNKALAAPIEKTISKAKGQPREPQVYTLPPSREEMTKNQVSLTCLVKGFYPSDIAVEWESNGQPENNYKTTPPVLDSDGSFFLYSKLTVDKSRWQQGNVFSCSVLHEALHSHYTQKSLSLSPG

SEQ ID NO: 51 - protein, 214 aa, synthetic construct
AIQMTQSPGTLSLSPGERATLSCRASQSVSSHLAWYQQKPGQAPRLLIYGASRRATGIPARFSGSGSGTDFTLTISRLEPEDFAVYYCQQYADSPLTFGQGTKVEIKRTVAAPSVFIFPPSDEQLKSGTASVVCLLNNFYPREAKVQWKVDNALQSGNSQESVTEQDSKDSTYSLSSTLTLSKADYEKHKVYACEVTHQGLSSPVTKSFNRGEC

SEQ ID NO: 52 - protein, 446 aa, synthetic construct
EVQLQESGPGLVKPSETLSLTCAVSGVSYSDYHWAWIRQPPGKGLEWIGDINHKGKTNYNPSLKSRVTISVDTSKNQFSLKLSSVTAADTAVYYCARDYPNFLFDYWGQGTLVTVSSASTKGPSVFPLAPSSKSTSGGTAALGCLVKDYFPEPVTVSWNSGALTSGVHTFPAVLQSSGLYSLSSVVTVPSSSLGTQTYICNVNHKPSNTKVDKKVEPKSCDKTHTCPPCPAPEAAGGPSVFLFPPKPKDTLMISRTPEVTCVVVDVSHEDPEVKFNWYVDGVEVHNAKTKPREEQYNSTYRVVSVLTVLHQDWLNGKEYKCKVSNKALAAPIEKTISKAKGQPREPQVYTLPPSREEMTKNQVSLTCLVKGFYPSDIAVEWESNGQPENNYKTTPPVLDSDGSFFLYSKLTVDKSRWQQGNVFSCSVLHEALHSHYTQKSLSLSPG

SEQ ID NO: 53 - protein, 214 aa, synthetic construct
DIQMTQSPATLSLSPGERATLSCRASQSVSTYLAWYQQKPGQAPRLLIYGASRRATGIPARFSGSGSGTDFTLTISSLQSEDFAVYYCQQYGDTPLTFGQGTKVEIKRTVAAPSVFIFPPSDEQLKSGTASVVCLLNNFYPREAKVQWKVDNALQSGNSQESVTEQDSKDSTYSLSSTLTLSKADYEKHKVYACEVTHQGLSSPVTKSFNRGEC

SEQ ID NO: 54 - protein, 446 aa, synthetic construct
ELQLQESGPGLVKPSETLSLTCAVSGISFNDFHWAWIRQPPGKGLEWIGDINHRGHTSYNPSLKSRVTVSVDTSKNQFSLKLSSVTAADTAVYYCARDYPNFTFDLWGQGTLVTVSSASTKGPSVFPLAPSSKSTSGGTAALGCLVKDYFPEPVTVSWNSGALTSGVHTFPAVLQSSGLYSLSSVVTVPSSSLGTQTYICNVNHKPSNTKVDKKVEPKSCDKTHTCPPCPAPEAAGGPSVFLFPPKPKDTLMISRTPEVTCVVVDVSHEDPEVKFNWYVDGVEVHNAKTKPREEQYNSTYRVVSVLTVLHQDWLNGKEYKCKVSNKALAAPIEKTISKAKGQPREPQVYTLPPSREEMTKNQVSLTCLVKGFYPSDIAVEWESNGQPENNYKTTPPVLDSDGSFFLYSKLTVDKSRWQQGNVFSCSVLHEALHSHYTQKSLSLSPG

SEQ ID NO: 55 - protein, 214 aa, synthetic construct
DIQLTQSPGTLSLSPGERATLSCRASQSVSSYLAWYQQKPGQAPRLLIYGASKRATGIPDRFSGSGSGTDFTLTISRLEPEDFAVYYCQQYGDSPLTFGQGTKVEIKRTVAAPSVFIFPPSDEQLKSGTASVVCLLNNFYPREAKVQWKVDNALQSGNSQESVTEQDSKDSTYSLSSTLTLSKADYEKHKVYACEVTHQGLSSPVTKSFNRGEC

SEQ ID NO: 56 - protein, 446 aa, synthetic construct
ELQLQESGPGLVKPSETLSLTCAVSGVSFSDYHWAWIRQPPGKGLEWIGDINHRGHTNYNPSLKSRVTVSIDTSKNQFSLKLSSVTAADTAVYFCARDFPNFIFDYWGQGTLVTVSSASTKGPSVFPLAPSSKSTSGGTAALGCLVKDYFPEPVTVSWNSGALTSGVHTFPAVLQSSGLYSLSSVVTVPSSSLGTQTYICNVNHKPSNTKVDKKVEPKSCDKTHTCPPCPAPEAAGGPSVFLFPPKPKDTLMISRTPEVTCVVVDVSHEDPEVKFNWYVDGVEVHNAKTKPREEQYNSTYRVVSVLTVLHQDWLNGKEYKCKVSNKALAAPIEKTISKAKGQPREPQVYTLPPSREEMTKNQVSLTCLVKGFYPSDIAVEWESNGQPENNYKTTPPVLDSDGSFFLYSKLTVDKSRWQQGNVFSCSVLHEALHSHYTQKSLSLSPG

SEQ ID NO: 57 - protein, 214 aa, synthetic construct
DIQLTQSPGTLSLSPGERATLSCRASQSVSTYLAWYQQKPGQAPRLLIYGASKRATGIPDRFSGSGSGTDFTLTISRLEPEDFAVYYCQQYGDSPLTFGQGTKVEIKRTVAAPSVFIFPPSDEQLKSGTASVVCLLNNFYPREAKVQWKVDNALQSGNSQESVTEQDSKDSTYSLSSTLTLSKADYEKHKVYACEVTHQGLSSPVTKSFNRGEC

SEQ ID NO: 58 - protein, 446 aa, synthetic construct
ELQLQESGPGLVKPSETLSLTCAVSGVSFSDYHWAWIRQPPGKGLEWIGDINHRGHTNYNPSLKSRVTVSIDTSKNQFSLKLSSVTAADTAVYFCARDFPNFIFDFWGQGTLVTVSSASTKGPSVFPLAPSSKSTSGGTAALGCLVKDYFPEPVTVSWNSGALTSGVHTFPAVLQSSGLYSLSSVVTVPSSSLGTQTYICNVNHKPSNTKVDKKVEPKSCDKTHTCPPCPAPEAAGGPSVFLFPPKPKDTLMISRTPEVTCVVVDVSHEDPEVKFNWYVDGVEVHNAKTKPREEQYNSTYRVVSVLTVLHQDWLNGKEYKCKVSNKALAAPIEKTISKAKGQPREPQVYTLPPSREEMTKNQVSLTCLVKGFYPSDIAVEWESNGQPENNYKTTPPVLDSDGSFFLYSKLTVDKSRWQQGNVFSCSVLHEALHSHYTQKSLSLSPG

SEQ ID NO: 59 - protein, 214 aa, synthetic construct
DIQLTQSPGTLSLSPGERATLSCRASQSVSNYLAWYQQKPGQAPRLLIYGASRRATGIPARFSGSGSGTDFTLTISSLEPEDFAVYYCQQYAASPLTFGQGTKVEIKRTVAAPSVFIFPPSDEQLKSGTASVVCLLNNFYPREAKVQWKVDNALQSGNSQESVTEQDSKDSTYSLSSTLTLSKADYEKHKVYACEVTHQGLSSPVTKSFNRGEC

SEQ ID NO: 60 - protein, 446 aa, synthetic construct
ELQLQESGPGLVKPSETLSLTCAVSGVSFTDYHWAWIRQPPGKGLEWIGDINHRGHTNYNPSLKSRVTVSIDTSKNQFSLKLSSVTAADTAVYYCARDYPNFIYDYWGQGTLVTVSSASTKGPSVFPLAPSSKSTSGGTAALGCLVKDYFPEPVTVSWNSGALTSGVHTFPAVLQSSGLYSLSSVVTVPSSSLGTQTYICNVNHKPSNTKVDKKVEPKSCDKTHTCPPCPAPEAAGGPSVFLFPPKPKDTLMISRTPEVTCVVVDVSHEDPEVKFNWYVDGVEVHNAKTKPREEQYNSTYRVVSVLTVLHQDWLNGKEYKCKVSNKALAAPIEKTISKAKGQPREPQVYTLPPSREEMTKNQVSLTCLVKGFYPSDIAVEWESNGQPENNYKTTPPVLDSDGSFFLYSKLTVDKSRWQQGNVFSCSVLHEALHSHYTQKSLSLSPG

SEQ ID NO: 61 - protein, 226 aa, synthetic construct
DKTHTCPPCPAPEAAGGPSVFLFPPKPKDTLMISRTPEVTCVVVDVSHEDPEVKFNWYVDGVEVHNAKTKPREEQYNSTYRVVSVLTVLHQDWLNGKEYKCKVSNKALGAPIEKTISKAKGQPREPQVCTLPPSREEMTKNQVSLSCAVKGFYPSDIAVEWESNGQPENNYKTTPPVLDSDGSFFLVSKLTVDKSRWQQGNVFSCSVMHEALHNHYTQKSLSLSPG

SEQ ID NO: 62 - protein, 446 aa, synthetic construct
ELQLQESGPGLVKPSETLSLTCAVSGLSFTDFYWAWIRQPPGKGLEWIGEINHKGNTSYNPSLKSRVTVSIDTSKNQFSLKLSSVTAADTAVYFCARDFPNYTFDFWGQGTLVTVSSASTKGPSVFPLAPSSKSTSGGTAALGCLVKDYFPEPVTVSWNSGALTSGVHTFPAVLQSSGLYSLSSVVTVPSSSLGTQTYICNVNHKPSNTKVDKKVEPKSCDKTHTCPPCPAPEAAGGPSVFLFPPKPKDTLMISRTPEVTCVVVDVSHEDPEVKFNWYVDGVEVHNAKTKPREEQYNSTYRVVSVLTVLHQDWLNGKEYKCKVSNKALGAPIEKTISKAKGQPREPQVYTLPPCREEMTKNQVSLWCLVKGFYPSDIAVEWESNGQPENNYKTTPPVLDSDGSFFLYSKLTVDKSRWQQGNVFSCSVMHEALHNHYTQKSLSLSPG

SEQ ID NO: 63 - protein, 446 aa, synthetic construct
EVQLQESGPGLVKPSETLSLTCAVSGVSYSDYHWAWIRQPPGKGLEWIGDINHKGKTNYNPSLKSRVTISVDTSKNQFSLKLSSVTAADTAVYYCARDYPNFLFDYWGQGTLVTVSSASTKGPSVFPLAPSSKSTSGGTAALGCLVKDYFPEPVTVSWNSGALTSGVHTFPAVLQSSGLYSLSSVVTVPSSSLGTQTYICNVNHKPSNTKVDKKVEPKSCDKTHTCPPCPAPEAAGGPSVFLFPPKPKDTLMISRTPEVTCVVVDVSHEDPEVKFNWYVDGVEVHNAKTKPREEQYNSTYRVVSVLTVLHQDWLNGKEYKCKVSNKALGAPIEKTISKAKGQPREPQVYTLPPCREEMTKNQVSLWCLVKGFYPSDIAVEWESNGQPENNYKTTPPVLDSDGSFFLYSKLTVDKSRWQQGNVFSCSVMHEALHNHYTQKSLSLSPG

SEQ ID NO: 64 - protein, 446 aa, synthetic construct
ELQLQESGPGLVKPSETLSLTCAVSGISFNDFHWAWIRQPPGKGLEWIGDINHRGHTSYNPSLKSRVTVSVDTSKNQFSLKLSSVTAADTAVYYCARDYPNFTFDLWGQGTLVTVSSASTKGPSVFPLAPSSKSTSGGTAALGCLVKDYFPEPVTVSWNSGALTSGVHTFPAVLQSSGLYSLSSVVTVPSSSLGTQTYICNVNHKPSNTKVDKKVEPKSCDKTHTCPPCPAPEAAGGPSVFLFPPKPKDTLMISRTPEVTCVVVDVSHEDPEVKFNWYVDGVEVHNAKTKPREEQYNSTYRVVSVLTVLHQDWLNGKEYKCKVSNKALGAPIEKTISKAKGQPREPQVYTLPPCREEMTKNQVSLWCLVKGFYPSDIAVEWESNGQPENNYKTTPPVLDSDGSFFLYSKLTVDKSRWQQGNVFSCSVMHEALHNHYTQKSLSLSPG

SEQ ID NO: 65 - protein, 446 aa, synthetic construct
ELQLQESGPGLVKPSETLSLTCAVSGVSFSDYHWAWIRQPPGKGLEWIGDINHRGHTNYNPSLKSRVTVSIDTSKNQFSLKLSSVTAADTAVYFCARDFPNFIFDYWGQGTLVTVSSASTKGPSVFPLAPSSKSTSGGTAALGCLVKDYFPEPVTVSWNSGALTSGVHTFPAVLQSSGLYSLSSVVTVPSSSLGTQTYICNVNHKPSNTKVDKKVEPKSCDKTHTCPPCPAPEAAGGPSVFLFPPKPKDTLMISRTPEVTCVVVDVSHEDPEVKFNWYVDGVEVHNAKTKPREEQYNSTYRVVSVLTVLHQDWLNGKEYKCKVSNKALGAPIEKTISKAKGQPREPQVYTLPPCREEMTKNQVSLWCLVKGFYPSDIAVEWESNGQPENNYKTTPPVLDSDGSFFLYSKLTVDKSRWQQGNVFSCSVMHEALHNHYTQKSLSLSPG

SEQ ID NO: 66 - protein, 446 aa, synthetic construct
ELQLQESGPGLVKPSETLSLTCAVSGVSFSDYHWAWIRQPPGKGLEWIGDINHRGHTNYNPSLKSRVTVSIDTSKNQFSLKLSSVTAADTAVYFCARDFPNFIFDFWGQGTLVTVSSASTKGPSVFPLAPSSKSTSGGTAALGCLVKDYFPEPVTVSWNSGALTSGVHTFPAVLQSSGLYSLSSVVTVPSSSLGTQTYICNVNHKPSNTKVDKKVEPKSCDKTHTCPPCPAPEAAGGPSVFLFPPKPKDTLMISRTPEVTCVVVDVSHEDPEVKFNWYVDGVEVHNAKTKPREEQYNSTYRVVSVLTVLHQDWLNGKEYKCKVSNKALGAPIEKTISKAKGQPREPQVYTLPPCREEMTKNQVSLWCLVKGFYPSDIAVEWESNGQPENNYKTTPPVLDSDGSFFLYSKLTVDKSRWQQGNVFSCSVMHEALHNHYTQKSLSLSPG

SEQ ID NO: 67 - protein, 446 aa, synthetic construct
ELQLQESGPGLVKPSETLSLTCAVSGVSFTDYHWAWIRQPPGKGLEWIGDINHRGHTNYNPSLKSRVTVSIDTSKNQFSLKLSSVTAADTAVYYCARDYPNFIYDYWGQGTLVTVSSASTKGPSVFPLAPSSKSTSGGTAALGCLVKDYFPEPVTVSWNSGALTSGVHTFPAVLQSSGLYSLSSVVTVPSSSLGTQTYICNVNHKPSNTKVDKKVEPKSCDKTHTCPPCPAPEAAGGPSVFLFPPKPKDTLMISRTPEVTCVVVDVSHEDPEVKFNWYVDGVEVHNAKTKPREEQYNSTYRVVSVLTVLHQDWLNGKEYKCKVSNKALGAPIEKTISKAKGQPREPQVYTLPPCREEMTKNQVSLWCLVKGFYPSDIAVEWESNGQPENNYKTTPPVLDSDGSFFLYSKLTVDKSRWQQGNVFSCSVMHEALHNHYTQKSLSLSPG

SEQ ID NO: 68 - protein, 251 aa, Homo sapiens
MAEDLGLSFGETASVEMLPEHGSCRPKARSSSARWALTCCLVLLPFLAGLTTYLLVSQLRAQGEACVQFQALKGQEFAPSHQQVYAPLRADGDKPRAHLTVVRQTPTQHFKNQFPALHWEHELGLAFTKNRMNYTNKFLLIPESGDYFIYSQVTFRGMTSECSEIRQAGRPNKPDSITVVITKVTDSYPEPTQLLMGTKSVCEVGSNWFQPIYLGAMFSLQEGDKLMVNVSDISLVDYTKEDKTFFGAFLL